European Patent Specification EP 4 071 171 B1, published June 25, 2025. Title: ANTI-TM4SF4 ANTIBODIES AND USE THEREOF. Applicant: Korea Atomic Energy Research Institute. The sequence listing filed with the application follows.

SEQUENCE LISTING (31 sequences)

SEQ ID NO: 1 - protein, 202 aa, Artificial Sequence
  TM4SF4
MCTGGCARCLGGTLIPLAFFGFLANILLFFPGGKVIDDNDHLSQEIWFFGGILGSGVLMIFPALVFLGLKNNDCCGCCGNEGCGKRFAMFTSTIFAVVGFLGAGYSFIISAISINKGPKCLMANSTWGYPFHDGDYLNDEALWNKCREPLNVVPWNLTLFSILLVVGGIQMVLCAIQVVNGLLGTLCGDCQCCGCCGGDGPV

SEQ ID NO: 2 - protein, 15 aa, Artificial Sequence
  epitope
TWGYPFHDGDYLNDE

SEQ ID NO: 3 - protein, 7 aa, Artificial Sequence
  ECL-2B7 CDR-H1
TYGIGVS

SEQ ID NO: 4 - protein, 16 aa, Artificial Sequence
  ECL-2B7 CDR-H2
HIWWNDNKYYNTALKS

SEQ ID NO: 5 - protein, 10 aa, Artificial Sequence
  ECL-2B7 CDR-H3
KEGSSAPFAY

SEQ ID NO: 6 - protein, 17 aa, Artificial Sequence
  ECL-2B7 CDR-L1
KSSQSLLNSSNQKNYLA

SEQ ID NO: 7 - protein, 7 aa, Artificial Sequence
  ECL-2B7 CDR-L2
FASTRES

SEQ ID NO: 8 - protein, 9 aa, Artificial Sequence
  ECL-2B7 CDR-L3
QQHYRTPPT

SEQ ID NO: 9 - protein, 7 aa, Artificial Sequence
  ECL-4C1 CDR-H1
TYGLGVG

SEQ ID NO: 10 - protein, 16 aa, Artificial Sequence
  ECL-4C1 CDR-H2
HIWWNDNKYYNTALKS

SEQ ID NO: 11 - protein, 10 aa, Artificial Sequence
  ECL-4C1 CDR-H3
KEGTSAPFAF

SEQ ID NO: 12 - protein, 17 aa, Artificial Sequence
  ECL-4C1 CDR-L1
KSSQSLLNGSNQKQYLA

SEQ ID NO: 13 - protein, 7 aa, Artificial Sequence
  ECL-4C1 CDR-L2
FASTRES

SEQ ID NO: 14 - protein, 9 aa, Artificial Sequence
  ECL-4C1 CDR-L3
QQHYRTPPT

SEQ ID NO: 15 - protein, 120 aa, Artificial Sequence
  ECL-2B7 Heavy chain variable region
EVKLEESGPGILQPSQTLSLTCSFSGFSLSTYGIGVSWIRQPSGKGLEWLAHIWWNDNKYYNTALKSRLTISKDTSNNQVFLKIASVDTADTATYYCARKEGSSAPFAYWGQGTLVTVSA

SEQ ID NO: 16 - protein, 114 aa, Artificial Sequence
  ECL-2B7 kappa chain variable region
DIVMTQSPSSLAMSVGQKVTMSCKSSQSLLNSSNQKNYLAWYQQKPGQSPKLLIYFASTRESGVPDRFIGSGSGTDFTLTISSMQAEDLADYFCQQHYRTPPTFGGGTKLEIKR

SEQ ID NO: 17 - DNA, 360 bp, Artificial Sequence
  ECL-2B7 Heavy chain variable region
gaggtgaagctggaggagtctggccctgggatattgcagccctcccagaccctcagtctgacttgttctttctctgggttttcactgagcacttatggtataggagtaagctggattcgtcagccttctgggaagggtctggagtggctggcacacatttggtggaatgataataagtactataacacagccctgaagagccggctcacaatctccaaggatacctccaacaaccaggtattcctcaagatcgccagtgtggacactgcagatactgccacatactactgtgctcgaaaggagggcagctcggccccctttgcttactggggccaagggactctggtcactgtctctgca

SEQ ID NO: 18 - DNA, 342 bp, Artificial Sequence
  ECL-2B7 kappa chain variable region
gatattgtgatgacccagtctccatcctccctggctatgtcagtaggacagaaggtcactatgagctgcaagtccagtcagagccttttaaatagtagcaatcaaaagaactatttggcctggtaccagcagaaaccaggacagtctcctaaacttctgatatactttgcatccactagggaatctggggtccctgatcgcttcataggcagtggatctgggacagatttcactcttaccatcagcagtatgcaggctgaagacctggcagattacttctgtcagcaacattatagaactcctccgacgttcggtggaggcaccaagctggaaatcaaacgg

SEQ ID NO: 19 - protein, 120 aa, Artificial Sequence
  ECL-4C1 Heavy chain variable region
EVKLEESGPGILQPSQTLSLTCSFSGFSLTTYGLGVGWIRQPSGKGLEWLAHIWWNDNKYYNTALKSRLTISKDTADTATYYCAASVDTADTATYYCARKEGTSAPFAFWGQGTLVTVSA

SEQ ID NO: 20 - protein, 114 aa, Artificial Sequence
  ECL-4C1 kappa chain variable region
DIVMTQSPSSLAMSVGERVTMSCKSSQSLLNGSNQKQYLAWFQQKPGQSPKLLVYFASTRESGVPDRFIGSGSGTDFTLTISSVQAEDLADYFCQQHYRTPPTFGGGTKLEIKR

SEQ ID NO: 21 - DNA, 360 bp, Artificial Sequence
  ECL-4C1 Heavy chain variable region
gaagttaagctggaggagtctggccctgggatattgcagccctcccagaccctcagtctgacttgttctttctctgggttttcactgaccacttatggtttaggagtaggctggattcgtcagccttcagggaagggtctggagtggctggcacacatttggtggaatgataataagtattataacacagccctgaagagccggctcacaatctccaaggatacctccaacaatcaggtattcctcaagatcgccagtgtggacactgcagatactgccacatactactgtgctcgaaaggagggcacctcggccccctttgctttctggggccaagggactctggtcactgtctctgca

SEQ ID NO: 22 - DNA, 341 bp, Artificial Sequence
  ECL-4C1 kappa chain variable region
gatattgtgatgacccagtctccatcctccctggctatgtcagtcggacagagggtcactatgagctgcaagtccagtcagagccttttaaatggtagcaatcaaaagaactatttggcctggttccagcagaaaccaggacagtctcctaaacttctggtatactttgcatccactagggaatctggggtccctgatcgcttcataggcagtggatctgggacagatttcactcttaccatcagcagtgtgcaggctgaagacctggcagattacttctgtcagcaacattataggactcctccgacgttcggtggaggcaccaagctggaaataaacgg

SEQ ID NO: 23 - protein, 30 aa, Artificial Sequence
  epitope
GGCARCLGGTLIPLAFFGFLANILLFFPGG

SEQ ID NO: 24 - protein, 15 aa, Artificial Sequence
  epitope
LGSGVLMIFPALVFL

SEQ ID NO: 25 - protein, 10 aa, Artificial Sequence
  epitope
NNDCCGCCGN

SEQ ID NO: 26 - protein, 21 aa, Artificial Sequence
  epitope
STIFAVVGFLGAGYSFIISAI

SEQ ID NO: 27 - protein, 7 aa, Artificial Sequence
  epitope
WGYPFHD

SEQ ID NO: 28 - protein, 7 aa, Artificial Sequence
  epitope
KGPKCLM

SEQ ID NO: 29 - protein, 53 aa, Artificial Sequence
  epitope
CREPLNVVPWNLTLFSILLVVGGIQMVLCAIQVVNGLLGTLCGDCQCCGCCGG

SEQ ID NO: 30 - RNA, 25 nt, Artificial Sequence
  TM4SF4 siRNA- sense
gccucucaaugugguucccuggaau

SEQ ID NO: 31 - RNA, 25 nt, Artificial Sequence
  TM4SF4 siRNA- antisense
auuccagggaaccacauugagaggc